European Patent Application EP 4 717 706 A1, published April 1, 2026. Title: Modified recombinant adeno-associated virus (AAV) binding protein and method for purification of AAV. Applicant: 東ソー株式会社. The sequence listing filed with the application follows.

SEQUENCE LISTING (61 sequences)

SEQ ID NO: 1 - protein, 1049 aa, Homo sapiens
  source 1..1049: note = KIAA0319L; note = UniProt No. Q8IZA0
MEKRLGVKPNPASWILSGYYWQTSAKWLRSLYLFYTCFCFSVLWLSTDASESRCQQGKTQFGVGLRSGGENHLWLLEGTPSLQSCWAACCQDSACHVFWWLEGMCIQADCSRPQSCRAFRTHSSNSMLVFLKKFQTADDLGFLPEDDVPHLLGLGWNWASWRQSPPRAALRPAVSSSDQQSLIRKLQKRGSPSDVVTPIVTQHSKVNDSNELGGLTTSGSAEVHKAITISSPLTTDLTAELSGGPKNVSVQPEISEGLATTPSTQQVKSSEKTQIAVPQPVAPSYSYATPTPQASFQSTSAPYPVIKELVVSAGESVQITLPKNEVQLNAYVLQEPPKGETYTYDWQLITHPRDYSGEMEGKHSQILKLSKLTPGLYEFKVIVEGQNAHGEGYVNVTVKPEPRKNRPPIAIVSPQFQEISLPTTSTVIDGSQSTDDDKIVQYHWEELKGPLREEKISEDTAILKLSKLVPGNYTFSLTVVDSDGATNSTTANLTVNKAVDYPPVANAGPNQVITLPQNSITLFGNQSTDDHGITSYEWSLSPSSKGKVVEMQGVRTPTLQLSAMQEGDYTYQLTVTDTIGQQATAQVTVIVQPENNKPPQADAGPDKELTLPVDSTTLDGSKSSDDQKIISYLWEKTQGPDGVQLENANSSVATVTGLQVGTYVFTLTVKDERNLQSQSSVNVIVKEEINKPPIAKITGNVVITLPTSTAELDGSKSSDDKGIVSYLWTRDEGSPAAGEVLNHSDHHPILFLSNLVEGTYTFHLKVTDAKGESDTDRTTVEVKPDPRKNNLVEIILDINVSQLTERLKGMFIRQIGVLLGVLDSDIIVQKIQPYTEQSTKMVFFVQNEPPHQIFKGHEVAAMLKSELRKQKADFLIFRALEVNTVTCQLNCSDHGHCDSFTKRCICDPFWMENFIKVQLRDGDSNCEWSVLYVIIATFVIVVALGILSWTVICCCKRQKGKPKRKSKYKILDATDQESLELKPTSRAGIKQKGLLLSSSLMHSESELDSDDAIFTWPDREKGKLLHGQNGSVPNGQTPLKARSPREEIL

SEQ ID NO: 2 - protein, 219 aa, synthetic construct
  source 1..219: note = AVR21
MKYLLPTAAAGLLLLAAQPAMAMGSAGESDQITLPKHEAQLNVYVLLVPPKGEASTYDWQLITHPRDYSGEMEGEHSQILKLSNLTPGLYEYRAVVEGQNAHSEGYVNVTVEPEPRKNRPPIAIVSPQFQEISLPTTSTVIDGSQSTDDDKIVQYHWEELKGPLREEKISEDTAILKLSQLVPGNYTFRLTVVDTDGATDSTTADLTVNKAVDHHHHHH

SEQ ID NO: 3 - DNA, 20 bp, synthetic construct
  source 1..20: mol_type = other DNA; note = T7 forward primer
taatacgactcactataggg

SEQ ID NO: 4 - DNA, 21 bp, synthetic construct
  source 1..21: mol_type = other DNA; note = T7 reverse primer
atgctagttattgctcagcgg

SEQ ID NO: 5 - protein, 219 aa, synthetic construct
  source 1..219: note = AVR24a
MKYLLPTAAAGLLLLAAQPAMAMGSAGESDQITLPKHEAQLKVYVLLVPPKGEASTYDWQLITHPRDYSGEMEGEHSQILKLSNLTPGLYEYRAVVEGQNAHSEGYVNVTVEPGPRKNRPPIAIVSPQFQEISLPTTSAVIDGSQSTDDDKIVQYHWEELKGPLREEKISEDTAILKLSQLVPGNYTFRLTVVDTDGATDSTTADLTVNKAVDHHHHHH

SEQ ID NO: 6 - protein, 219 aa, synthetic construct
  source 1..219: note = AVR24b
MKYLLPTAAAGLLLLAAQPAMAMGSAGESDQITLPKHEAQLNVYVLLVPPRGEASTYDWQLITHPRDYSGEMEGEHSQILKLSNLTPGLYEYRAVVEGQNAHSEGYVNVTVEPEPRKNRPPIAIVSPQFQEISLPTTSAVIDGSQSTDDDKIVQYHWEELKGPLREEKISEDTPILKLSQLVPGNYTFRLTVVDTDGATDSTTADLTVNKAVDHHHHHH

SEQ ID NO: 7 - protein, 219 aa, synthetic construct
  source 1..219: note = AVR25a
MKYLLPTAAAGLLLLAAQPAMAMGSAGESDQITLPKHEAQLKVYVLLVPPKGEASTYDWQLITHPRDYSGEMEGEHSQILKLSNLTPGLYEYRAVVEGQNAHSEGYVNVTVEPGPRKNRPPIAIVSPQFQEISLPTTSAVIDGSQSTDDDKIVQYHWEELKGPLREEKISEDTPILKLSQLVPGNYTFRLTVVDTDGATDSTTADLTVNKAVDHHHHHH

SEQ ID NO: 8 - protein, 219 aa, synthetic construct
  source 1..219: note = AVR25b
MKYLLPTAAAGLLLLAAQPAMAMGSAGESDQITLPKHEAQLNVYVLLVPPRGEASTYDWQLITHPRDYSGEMEGEHSQILKLSNLTPGLYEYRAVVEGQNAHSEGYVNVTVEPGPRKNRPPIAIVSPQFQEISLPTTSAVIDGSQSTDDDKIVQYHWEELKGPLREEKISEDTPILKLSQLVPGNYTFRLTVVDTDGATDSTTADLTVNKAVDHHHHHH

SEQ ID NO: 9 - protein, 219 aa, synthetic construct
  source 1..219: note = AVR26
MKYLLPTAAAGLLLLAAQPAMAMGSAGESDQITLPKHEAQLKVYVLLVPPRGEASTYDWQLITHPRDYSGEMEGEHSQILKLSNLTPGLYEYRAVVEGQNAHSEGYVNVTVEPGPRKNRPPIAIVSPQFQEISLPTTSAVIDGSQSTDDDKIVQYHWEELKGPLREEKISEDTPILKLSQLVPGNYTFRLTVVDTDGATDSTTADLTVNKAVDHHHHHH

SEQ ID NO: 10 - DNA, 25 bp, synthetic construct
  source 1..25: mol_type = other DNA; note = N329K forward primer
agctgaaagtctacgtactgctggt

SEQ ID NO: 11 - DNA, 25 bp, synthetic construct
  source 1..25: mol_type = other DNA; note = N329K reverse primer
tagactttcagctgggcttcatgtt

SEQ ID NO: 12 - DNA, 25 bp, synthetic construct
  source 1..25: mol_type = other DNA; note = K338R forward primer
caccgcgcggggaagcgtcaacgta

SEQ ID NO: 13 - DNA, 25 bp, synthetic construct
  source 1..25: mol_type = other DNA; note = K338R reverse primer
tccccgcgcggtggaaccagcagta

SEQ ID NO: 14 - DNA, 25 bp, synthetic construct
  source 1..25: mol_type = other DNA; note = E401G forward primer
agcctggcccgcgcaagaatcgtcc

SEQ ID NO: 15 - DNA, 25 bp, synthetic construct
  source 1..25: mol_type = other DNA; note = E401G reverse primer
cgcgggccaggctcaaccgttacgt

SEQ ID NO: 16 - DNA, 25 bp, synthetic construct
  source 1..25: mol_type = other DNA; note = T426A forward primer
caagtgcggtgatcgacggatcgca

SEQ ID NO: 17 - DNA, 25 bp, synthetic construct
  source 1..25: mol_type = other DNA; note = T426A reverse primer
atcaccgcacttgtagtcgggagtg

SEQ ID NO: 18 - DNA, 25 bp, synthetic construct
  source 1..25: mol_type = other DNA; note = A461P forward primer
ataccccgattcttaagctctcgca

SEQ ID NO: 19 - DNA, 25 bp, synthetic construct
  source 1..25: mol_type = other DNA; note = A461P reverse primer
agaatcggggtatcctcgctgatct

SEQ ID NO: 20 - protein, 239 aa, synthetic construct
  source 1..239: note = Enhanced green fluorescence protein(EGFP)
MVSKGEELFTGVVPILVELDGDVNGHKFSVSGEGEGDATYGKLTLKFICTTGKLPVPWPTLVTTLTYGVQCFSRYPDHMKQHDFFKSAMPEGYVQERTIFFKDDGNYKTRAEVKFEGDTLVNRIELKGIDFKEDGNILGHKLEYNYNSHNVYIMADKQKNGIKVNFKIRHNIEDGSVQLADHYQQNTPIGDGPVLLPDNHYLSTQSALSKDPNEKRDHMVLLEFVTAAGITLGMDELYK

SEQ ID NO: 21 - DNA, 732 bp, synthetic construct
  source 1..732: mol_type = other DNA; note = EGFP DNA
gaattcatggtgagcaaaggcgaggaactgtttactggtgtagtccccatactggtggaacttgatggggatgtcaatggtcacaaatttagcgtgtcaggagaaggcgaaggagatgcgacgtacggcaagctgacccttaagttcatctgtaccacgggtaagttgcctgttccttggcccacacttgtgacaaccctgacctatggagtgcaatgcttctccagatatccagaccacatgaagcagcatgacttcttcaaatccgccatgccagaaggctatgtgcaggaaaggaccatcttctttaaggacgacggaaactacaaaactcgtgctgaggtgaagttcgaaggagacacactggtgaatcgaatcgagctgaaagggattgactttaaggaggacgggaatattctgggccataagctggagtacaactacaactctcacaatgtgtacatcatggccgacaaacagaagaacgggattaaggtcaactttaagattcgccacaacatcgaggatggtagtgtacagctcgctgaccattaccagcagaatactcccataggcgatggaccagttttgctgcctgacaaccattatctgtcaacccaatctgccctgagcaaagatccgaatgagaaacgggatcacatggttctcttggagtttgtcacagcagcagggatcactctcggcatggatgagctctataaatagggatcc

SEQ ID NO: 22 - protein, 219 aa, synthetic construct
  source 1..219: note = AVR8g
MKYLLPTAAAGLLLLAAQPAMAMGSAGESDQITLPKNEVQLNAYVLQEPPKGETCTYDWQLITHPRDYSGEMEGEHSQILKLSNLTPGLYEFKVIVEGQNAHSEGYVNVTVEPEPRKNRPPIAIVSPQFQEISLPTTSTVIDGSQSTDDDKIVQYHWEELKGPLREEKISEDTAILKLSKLVPGNYTFRLTVVDSDGATDSTTANLTVNKAVDHHHHHH

SEQ ID NO: 23 - DNA, 657 bp, synthetic construct
  source 1..657: mol_type = other DNA; note = AVR8g DNA
atgaaatacctgctgccgaccgctgctgctggtctgctgctcctcgctgcccagccggcgatggccatgggctctgcaggcgagtcggatcagattaccctgccgaagaacgaagtacaactgaatgcgtatgtgctgcaggaaccaccgaaaggggaaacctgtacgtatgactggcagcttattacgcatcctcgcgactacagcggcgagatggaaggagaacattcgcagattctgaaactgtccaatctgacgccgggtctgtatgaattcaaggttatcgttgaaggtcagaatgcacatagcgaaggctatgttaacgttaccgtggaaccggagccacgcaagaaccgtcctccgatcgccattgtttcaccgcagtttcaggagatttcactgccgaccaccagtaccgttatcgatggttcgcagtcaacggatgacgacaaaatcgttcagtaccactgggaagagctgaaaggccccttacgcgaagagaagatcagcgaagataccgccatcttgaaattatcgaaacttgtgccgggtaattacacgttcagactgacggtggtcgattctgatggcgcaaccgactccaccaccgccaaccttaccgtcaacaaagcggtagaccatcatcatcatcatcat

SEQ ID NO: 24 - protein, 219 aa, synthetic construct
  source 1..219: note = AVR9a
MKYLLPTAAAGLLLLAAQPAMAMGSAGESDQITLPKNEVQLNAHVLQEPPKGETCTYDWQLITHPRDYSGEMEGEHSQILKLSNLTPGLYEFKVIVEGQNAHSEGYVNVTVEPEPRKNRPPIAIVSPQFQEISLPTTSTVIDGSQSTDDDKIVQYHWEELKGPLREEKISEDTAILKLSKLVPGNYTFRLTVVDSDGATDSTTANLTVNKAVDHHHHHH

SEQ ID NO: 25 - protein, 219 aa, synthetic construct
  source 1..219: note = AVR9b
MKYLLPTAAAGLLLLAAQPAMAMGSAGESDQITLPKNEVQLNAYVLQEPPKGETCTYDWQLITHPRDYSGEMEGEHSQILKLSNLTPGLYESKVIVEGQNAHSEGYVNVTVEPEPRKNRPPIAIVSPQFQEISLPTTSTVIDGSQSTDDDKIVQYHWEELKGPLREEKISEDTAILKLSKLVPGNYTFRLTVVDSDGATDSTTANLTVNKAVDHHHHHH

SEQ ID NO: 26 - protein, 219 aa, synthetic construct
  source 1..219: note = AVR9c
MKYLLPTAAAGLLLLAAQPAMAMGSAGESDQITLPKNEVQLNAYVLQEPPKGETCTYDWQLITHPRDYSGEMEGEHSQILKLSNLTPGLYEFKVIVEGQNAHSEGYVNVTVEPEPRKNRPPIAIVSPQFQEISLPTTSTVIDGSQSTDDDKIVQYHWEELKGPLREEKISEDTAILKLSNLVPGNYTFRLTVVDSDGATDSTTANLTVNKAVDHHHHHH

SEQ ID NO: 27 - protein, 219 aa, synthetic construct
  source 1..219: note = AVR9d
MKYLLPTAAAGLLLLAAQPAMAMGSAGESDQITLPKNEVQLNAYVLQEPPKGETCTYDWQLITHPRDYSGEMEGEHSQILKLSNLTPGLYEFKVIVEGQNAHSEGYVNVTVEPEPRKNRPPIAIVSPQFQEISLPTTSTVIDGSQSTDDDKIVQYHWEELKGPLREEKISEDTAILKLSKLVPGNYTFRLTVVDSDGATDSTTTNLTVNKAVDHHHHHH

SEQ ID NO: 28 - protein, 219 aa, synthetic construct
  source 1..219: note = AVR25c
MKYLLPTAAAGLLLLAAQPAMAMGSAGESDQITLPKHEAQLKVYVLLVPPKGEASTYDWQLITHPRDYSGEMEGEHSQILKLSNLTPGLYEYRAVVEGQNAHSEGYVNVTVEPGPRKNRPPIAIVSPQFQEISLPTTSAVIDGSQSTDDDKIVQYHWEELKGPLREEKISEDTPILKLSNLVPGNYTFRLTVVDTDGATDSTTADLTVNKAVDHHHHHH

SEQ ID NO: 29 - DNA, 26 bp, synthetic construct
  source 1..26: mol_type = other DNA; note = K467N forward primer
gagagcttaagaatgggggtatcctc

SEQ ID NO: 30 - DNA, 25 bp, synthetic construct
  source 1..25: mol_type = other DNA; note = K467N reverse primer
ttcttaagctctcgaatctggtacc

SEQ ID NO: 31 - protein, 219 aa, synthetic construct
  source 1..219: note = AVR27b
MKYLLPTAAAGLLLLAAQPAMAMGSAGESDQITLPKHEAQLKVYVLLVPPKGEASTYDWQLITHPRDYSGEMEGEHSQFLKLSNLTPGLYEYRAVVEGQNAHSEGYVNVTVEPGPRKNRPPIAIVSPQFQEISLPTTSAVIDGSQSTDDDKIVQYHWEELKGPLREEKISEDTPILKLSNLVPGNYRFRLTVVDTDGATDSTTADLTVNKAVDHHHHHH

SEQ ID NO: 32 - protein, 219 aa, synthetic construct
  source 1..219: note = AVR27c
MKYLLPTAAAGLLLLAAQPAMAMGSAGESDQITLPKHEAQLKVYVLLVPPKGEASTYDWQLITHPRDYSGEMEGEHSQILKLSNLTPGLYEYRAVVEGQNAHSEGYANVTVEPGPRKNRPPIAIVSPQFQEISLPTTSAVIDGSQSTDDDKIVQYHWEELKGPLREEKISEDTPILKLSNLVPGNYRFRLTVVDTDGATDSTTADLTVNKAVDHHHHHH

SEQ ID NO: 33 - protein, 219 aa, synthetic construct
  source 1..219: note = AVR27d
MKYLLPTAAAGLLLLAAQPAMAMGSAGESDQITLPKHEAQLKVYVLLVPPKGEASTYDWQLITHPRDYSGEMEGEHSQILKLSNLTPGLYEYRAVVEGQNAHSEGYVNVTVEPGPRKNRPPIAIVSPQFQEISLPTTSAVIDGSQSTDDDKIVQYHWEELKGPLREERISEDTPILKLSNLVPGNYRFRLTVVDTDGATDSTTADLTVNKAVDHHHHHH

SEQ ID NO: 34 - protein, 219 aa, synthetic construct
  source 1..219: note = AVR28
MKYLLPTAAAGLLLLAAQPAMAMGSAGESDQITLPKHEAQLKVYVLLVPPKGEASTYDWQLITHPRDYSGEMEGEHSQFLKLSNLTPGLYEYRAVVEGQNAHSEGYANVTVEPGPRKNRPPIAIVSPQFQEISLPTTSAVIDGSQSTDDDKIVQYHWEELKGPLREERISEDTPILKLSNLVPGNYTFRLTVVDTDGATDSTTADLTVNKAVDHHHHHH

SEQ ID NO: 35 - protein, 219 aa, synthetic construct
  source 1..219: note = AVR29a
MKYLLPTAAAGLLLLAAQPAMAMGSAGESDQITLPKHEAQLKVYVLLVPPKGEASTYDWQLITHPRDYSGEMEGEHSQFLKLSNLTPGLYEYRAVVEGQNAHSEGYANVTVEPGPRKNRPPIAIVSPQFQEISLPTTSAVIDGSQSTDDDKIVQYHWEELKGPLREERISEDTPILKLSNLVPGNYRFRLTVVDTDGATDSTTADLTVNKAVDHHHHHH

SEQ ID NO: 36 - protein, 219 aa, synthetic construct
  source 1..219: note = AVR29b
MKYLLPTAAAGLLLLAAQPAMAMGSADESDQITLPKHEAQLKVYVLLVPPKGEASTYDWQLITHPRDYSGEMEGEHSQFLKLSNLTPGLYEYRAVVEGQNAHSEGYANVTVEPGPRKNRPPIAIVSPQFQEISLPTTSAVIDGSQSTDDDKIVQYHWEELKGPLREERISEDTPILKLSNLVPGNYTFRLTVVDTDGATDSTTADLTVNKAVDHHHHHH

SEQ ID NO: 37 - protein, 219 aa, synthetic construct
  source 1..219: note = AVR29c
MKYLLPTAAAGLLLLAAQPAMAMGSAGESDQITLPKHEAQLKVYVLLVPPKGEASTYDWQLITHPRDYSGEMEGEHSQFLKLSNLTPGLYEYRAVVEGQNAHSEGYANVTVEPGPRKNRPPIAIVSPQFQEISLPTTSAVIDGSQSTDDDKIVQYHWEELKGPLREERISEDTPILKLSNLVPGNYTFRLTVVDTDGATDSTTADLTVNEAVDHHHHHH

SEQ ID NO: 38 - protein, 219 aa, synthetic construct
  source 1..219: note = AVR29d
MKYLLPTAAAGLLLLAAQPAMAMGSAGESDQITLPKHEAQLKVYVLLVPPKGEASTYDWQLITHPRDYSGEMEGEHSQFLKLSNLTPGLYEYRAVVEGQNAHSEGYANVTVEPGPRKNRPPIAIVSPQFQEISLPTTSAVIDGSQSTDDDKIVQYHWEELKGPLREERISEDTPILKLSNLVPGNYTFRLTVVDTDGATDSTTADLTVNKAIDHHHHHH

SEQ ID NO: 39 - protein, 219 aa, synthetic construct
  source 1..219: note = AVR31
MKYLLPTAAAGLLLLAAQPAMAMGSADESDQITLPKHEAQLKVYVLLVPPKGEASTYDWQLITHPRDYSGEMEGEHSQFLKLSNLTPGLYEYRAVVEGQNAHSEGYANVTVEPGPRKNRPPIAIVSPQFQEISLPTTSAVIDGSQSTDDDKIVQYHWEELKGPLREERISEDTPILKLSNLVPGNYTFRLTVVDTDGATDSTTADLTVNEAIDHHHHHH

SEQ ID NO: 40 - DNA, 25 bp, synthetic construct
  source 1..25: mol_type = other DNA; note = G314D forward primer
ctgcagatgaaagcgaccaaatcac

SEQ ID NO: 41 - DNA, 25 bp, synthetic construct
  source 1..25: mol_type = other DNA; note = G314D reverse primer
ctttcatctgcagagcccatggcca

SEQ ID NO: 42 - DNA, 25 bp, synthetic construct
  source 1..25: mol_type = other DNA; note = I366F forward primer
gtcagtttctgaaattatccaactt

SEQ ID NO: 43 - DNA, 25 bp, synthetic construct
  source 1..25: mol_type = other DNA; note = I366F reverse primer
ttcagaaactgactgtgttcgcctt

SEQ ID NO: 44 - DNA, 25 bp, synthetic construct
  source 1..25: mol_type = other DNA; note = V394A forward primer
ggtatgcgaacgtaacggttgagcc

SEQ ID NO: 45 - DNA, 25 bp, synthetic construct
  source 1..25: mol_type = other DNA; note = V394A reverse primer
acgttcgcatacccctcggaatgcg

SEQ ID NO: 46 - DNA, 25 bp, synthetic construct
  source 1..25: mol_type = other DNA; note = K455R forward primer
aagaacgcatcagcgaggatacccc

SEQ ID NO: 47 - DNA, 25 bp, synthetic construct
  source 1..25: mol_type = other DNA; note = K455R reverse primer
ctgatgcgttcttcacggagcgggc

SEQ ID NO: 48 - DNA, 25 bp, synthetic construct
  source 1..25: mol_type = other DNA; note = T474R forward primer
actaccgctttcgcctgaccgtgac

SEQ ID NO: 49 - DNA, 25 bp, synthetic construct
  source 1..25: mol_type = other DNA; note = T474R reverse primer
cgaaagcggtagttacctggtacca

SEQ ID NO: 50 - DNA, 25 bp, synthetic construct
  source 1..25: mol_type = other DNA; note = K497E forward primer
ttaacgaagccgtcgaccatcatca

SEQ ID NO: 51 - DNA, 25 bp, synthetic construct
  source 1..25: mol_type = other DNA; note = K497E reverse primer
acggcttcgttaacggtcaagtctg

SEQ ID NO: 52 - DNA, 25 bp, synthetic construct
  source 1..25: mol_type = other DNA; note = V499I forward primer
aagccattgaccatcatcatcatca

SEQ ID NO: 53 - DNA, 25 bp, synthetic construct
  source 1..25: mol_type = other DNA; note = V499I reverse primer
tggtcaatggctttgttaacggtca

SEQ ID NO: 54 - DNA, 30 bp, synthetic construct
  source 1..30: mol_type = other DNA; note = K497E_V499I forward primer
aacgaagccattgaccatcatcatcatcat

SEQ ID NO: 55 - DNA, 30 bp, synthetic construct
  source 1..30: mol_type = other DNA; note = K497E_V499I reverse primer
gtcaatggcttcgttaacggtcaagtctgc

SEQ ID NO: 56 - DNA, 25 bp, synthetic construct
  source 1..25: mol_type = other DNA; note = AVR29c(-) forward primer
acatatgtctgcaggcgaaagcgac

SEQ ID NO: 57 - DNA, 26 bp, synthetic construct
  source 1..26: mol_type = other DNA; note = AVR29c(-) reverse primer
cctgcagacatatgtatatctccttc

SEQ ID NO: 58 - protein, 196 aa, synthetic construct
  source 1..196: note = AVR29c(-)
MSAGESDQITLPKHEAQLKVYVLLVPPKGEASTYDWQLITHPRDYSGEMEGEHSQFLKLSNLTPGLYEYRAVVEGQNAHSEGYANVTVEPGPRKNRPPIAIVSPQFQEISLPTTSAVIDGSQSTDDDKIVQYHWEELKGPLREERISEDTPILKLSNLVPGNYTFRLTVVDTDGATDSTTADLTVNEAVDHHHHHH

SEQ ID NO: 59 - DNA, 18 bp, synthetic construct
  source 1..18: mol_type = other DNA; note = Forward primer
ctccatcactaggggttc

SEQ ID NO: 60 - DNA, 18 bp, synthetic construct
  source 1..18: mol_type = other DNA; note = Reverse primer
ttgggattccaggcatgc

SEQ ID NO: 61 - DNA, 16 bp, synthetic construct
  source 1..16: mol_type = other DNA; note = Probe
tcccttccctgtcctt